European Patent Application EP 4 574 171 A1, published June 25, 2025. Title: Pharmaceutical composition for treating and/or preventing cystic kidney ciliopathy. Applicant: KYOTO UNIVERSITY. Application JP. The sequence listing filed with the application follows.

SEQUENCE LISTING (3 sequences)

SEQ ID NO: 1 - DNA, 57 bp, synthetic construct
  source 1..57: mol_type = other DNA
gagaccacttggatccgggatcaggtcttcatctaggttttagagctagaaatagca

SEQ ID NO: 2 - DNA, 20 bp, synthetic construct
  source 1..20: mol_type = other DNA
cgtccattgtgggtagcaat

SEQ ID NO: 3 - DNA, 20 bp, synthetic construct
  source 1..20: mol_type = other DNA
tctctgtcttctccccagga